European Patent Specification EP 4 001 302 B1, published June 21, 2023. Title: carrier peptide fragment and use thereof. Applicant: TOAGOSEI CO., LTD. The sequence listing filed with the application follows.

SEQUENCE LISTING (4 sequences)

SEQ ID NO: 1 - protein, 7 aa, Artificial Sequence
  synthetic peptide
VVRSLVK

SEQ ID NO: 2 - protein, 13 aa, Artificial Sequence
  synthetic peptide
KKRTLRKNDRKKR

SEQ ID NO: 3 - protein, 15 aa, Artificial Sequence
  synthetic peptide
TLKERCLQVVRSLVK

SEQ ID NO: 4 - protein, 14 aa, Artificial Sequence
  synthetic peptide
VVRSLVKVVRSLVK